European Patent Specification EP 3 394 263 B1, published February 26, 2025. Title: TLR inhibitory oligonucleotides and their use. Applicant: SBI Biotech Co., Ltd. The sequence listing filed with the application follows.

SEQUENCE LISTING (50 sequences)

SEQ ID NO: 1 - DNA, 18 bp, Artificial Sequence
  (CCT)6 inhibitory oligonucleotide
cctcctcctcctcctcct

SEQ ID NO: 2 - DNA, 21 bp, Artificial Sequence
  (CCT)7 inhibitory oligonucleotide
cctcctcctcctcctcctcct

SEQ ID NO: 3 - DNA, 24 bp, Artificial Sequence
  (CCT)8 inhibitory oligonucleotide
cctcctcctcctcctcctcctcct

SEQ ID NO: 4 - DNA, 25 bp, Artificial Sequence
  (CCT)8C inhibitory olionucleotide
cctcctcctcctcctcctcctcctc

SEQ ID NO: 5 - DNA, 26 bp, Artificial Sequence
  (CCT)8CC inhibitory oligonucleotide
cctcctcctcctcctcctcctcctcc

SEQ ID NO: 6 - DNA, 27 bp, Artificial Sequence
  (CCT)9 inhibitory oligonucleotide
cctcctcctcctcctcctcctcctcct

SEQ ID NO: 7 - DNA, 28 bp, Artificial Sequence
  Inhibitory oligonucleotide
cctcctcctcctcctcctcctcctcctc

SEQ ID NO: 8 - DNA, 29 bp, Artificial Sequence
  Inhibitory oligonucleotide
cctcctcctcctcctcctcctcctcctcc

SEQ ID NO: 9 - DNA, 30 bp, Artificial Sequence
  (CCT)10 inhibitory oligonucleotide
cctcctcctcctcctcctcctcctcctcct

SEQ ID NO: 10 - DNA, 31 bp, Artificial Sequence
  (CCT)10C inhibitory oligonucleotide
cctcctcctcctcctcctcctcctcctcctc

SEQ ID NO: 11 - DNA, 32 bp, Artificial Sequence
  (CCT)10CC inhibitory oligonucleotide
cctcctcctcctcctcctcctcctcctcctcc

SEQ ID NO: 12 - DNA, 33 bp, Artificial Sequence
  (CCT)11 inhibitory oligonucleotide
cctcctcctcctcctcctcctcctcctcctcct

SEQ ID NO: 13 - DNA, 34 bp, Artificial Sequence
  (CCT)11C inhibitory oligonucleotide
cctcctcctcctcctcctcctcctcctcctcctc

SEQ ID NO: 14 - DNA, 35 bp, Artificial Sequence
  (CCT)11CC inhibitory oligonucleotide
cctcctcctcctcctcctcctcctcctcctcctcc

SEQ ID NO: 15 - DNA, 36 bp, Artificial Sequence
  (CCT)12 inhibitory oligonucleotide
cctcctcctcctcctcctcctcctcctcctcctcct

SEQ ID NO: 16 - DNA, 42 bp, Artificial Sequence
  (CCT)14 inhibitory oligonucleotide
cctcctcctcctcctcctcctcctcctcctcctcctcctcct

SEQ ID NO: 17 - DNA, 48 bp, Artificial Sequence
  (CCT)16 inhibitory oligonucleotide
cctcctcctcctcctcctcctcctcctcctcctcctcctcctcctcct

SEQ ID NO: 18 - DNA, 18 bp, Artificial Sequence
  (TCC)6 inhibitory oligonucleotide
tcctcctcctcctcctcc

SEQ ID NO: 19 - DNA, 27 bp, Artificial Sequence
  (TCC)9 inhibitory oligonucleotide
tcctcctcctcctcctcctcctcctcc

SEQ ID NO: 20 - DNA, 36 bp, Artificial Sequence
  (TCC)12 inhibitory oligonucleotide
tcctcctcctcctcctcctcctcctcctcctcctcc

SEQ ID NO: 21 - DNA, 18 bp, Artificial Sequence
  Inhibitory oligonucleotide
  modified_base (1)..(8): phosphorothioate-modified at 3' internucleotide bond
  modified_base (10)..(17): phosphorothioate-modified at 3' internucleotide bond
cctcctcctcctcctcct

SEQ ID NO: 22 - DNA, 27 bp, Artificial Sequence
  Inhibitory oligonucleotide
  modified_base (1)..(8): phosphorothioate-modified at 3' internucleotide bond
  modified_base (10)..(17): phosphorothioate-modified at 3' internucleotide bond
  modified_base (19)..(26): phosphorothioate-modified at 3' internucleotide bond
cctcctcctcctcctcctcctcctcct

SEQ ID NO: 23 - DNA, 27 bp, Artificial Sequence
  Inhibitory oligonucleotide
  modified_base (1)..(5): phosphorothioate-modified at 3' internucleotide bond
  modified_base (7)..(14): phosphorothioate-modified at 3' internucleotide bond
  modified_base (16)..(23): phosphorothioate-modified at 3' internucleotide bond
  modified_base (25)..(26): phosphorothioate-modified at 3' internucleotide bond
cctcctcctcctcctcctcctcctcct

SEQ ID NO: 24 - DNA, 27 bp, Artificial Sequence
  Inhibitory oligonucleotide
  modified_base (1)..(2): phosphorothioate-modified at 3' internucleotide bond
  modified_base (4)..(11): phosphorothioate-modified at 3' internucleotide bond
  modified_base (13)..(20): phosphorothioate-modified at 3' internucleotide bond
  modified_base (22)..(26): phosphorothioate-modified at 3' internucleotide bond
cctcctcctcctcctcctcctcctcct

SEQ ID NO: 25 - DNA, 36 bp, Artificial Sequence; identical to SEQ ID NO: 15
  Inhibitory oligonucleotide
  modified_base (1)..(5): phosphorothioate-modified at 3' internucleotide bond
  modified_base (7)..(11): phosphorothioate-modified at 3' internucleotide bond
  modified_base (13)..(17): phosphorothioate-modified at 3' internucleotide bond
  modified_base (19)..(23): phosphorothioate-modified at 3' internucleotide bond
  modified_base (25)..(29): phosphorothioate-modified at 3' internucleotide bond
  modified_base (31)..(35): phosphorothioate-modified at 3' internucleotide bond

SEQ ID NO: 26 - DNA, 36 bp, Artificial Sequence; identical to SEQ ID NO: 15
  Inhibitory oligonucleotide
  modified_base (1)..(8): phosphorothioate-modified at 3' internucleotide bond
  modified_base (10)..(17): phosphorothioate-modified at 3' internucleotide bond
  modified_base (19)..(26): phosphorothioate-modified at 3' internucleotide bond
  modified_base (28)..(35): phosphorothioate-modified at 3' internucleotide bond

SEQ ID NO: 27 - DNA, 36 bp, Artificial Sequence; identical to SEQ ID NO: 15
  Inhibitory oligonculeotide
  modified_base (1)..(5): phosphorothioate-modified at 3' internucleotide bond
  modified_base (7)..(14): phosphorothioate-modified at 3' internucleotide bond
  modified_base (16)..(23): phosphorothioate-modified at 3' internucleotide bond
  modified_base (25)..(32): phosphorothioate-modified at 3' internucleotide bond
  modified_base (34)..(35): phosphorothioate-modified at 3' internucleotide bond

SEQ ID NO: 28 - DNA, 36 bp, Artificial Sequence; identical to SEQ ID NO: 15
  Inhibitory Oligonucleotide
  modified_base (1)..(2): phosphorothioate-modified at 3' internucleotide bond
  modified_base (4)..(11): phosphorothioate-modified at 3' internucleotide bond
  modified_base (13)..(20): phosphorothioate-modified at 3' internucleotide bond
  modified_base (22)..(29): phosphorothioate-modified at 3' internucleotide bond
  modified_base (31)..(35): phosphorothioate-modified at 3' internucleotide bond

SEQ ID NO: 29 - DNA, 18 bp, Artificial Sequence
  Inhibitory Oligonucleotide
  modified_base (1)..(8): phosphorothioate-modified at 3' internucleotide bond
  modified_base (10)..(17): phosphorothioate-modified at 3' internucleotide bond
ctcctcctcctcctcctc

SEQ ID NO: 30 - DNA, 27 bp, Artificial Sequence
  Inhibitory Oligonucleotide
  modified_base (1)..(8): phosphorothioate-modified at 3' internucleotide bond
  modified_base (10)..(17): phosphorothioate-modified at 3' internucleotide bond
  modified_base (19)..(26): phosphorothioate-modified at 3' internucleotide bond
ctcctcctcctcctcctcctcctcctc

SEQ ID NO: 31 - DNA, 27 bp, Artificial Sequence
  Inhibitory Oligonucleotide
  modified_base (1)..(5): phosphorothioate-modified at 3' internucleotide bond
  modified_base (7)..(14): phosphorothioate-modified at 3' internucleotide bond
  modified_base (16)..(23): phosphorothioate-modified at 3' internucleotide bond
  modified_base (25)..(26): phosphorothioate-modified at 3' internucleotide bond
ctcctcctcctcctcctcctcctcctc

SEQ ID NO: 32 - DNA, 27 bp, Artificial Sequence
  Inhibitory Oligonucleotide
  modified_base (1)..(2): phosphorothioate-modified at 3' internucleotide bond
  modified_base (4)..(11): phosphorothioate-modified at 3' internucleotide bond
  modified_base (13)..(20): phosphorothioate-modified at 3' internucleotide bond
  modified_base (22)..(26): phosphorothioate-modified at 3' internucleotide bond
ctcctcctcctcctcctcctcctcctc

SEQ ID NO: 33 - DNA, 36 bp, Artificial Sequence
  Inhibitory Oligonucleotide
  modified_base (1)..(8): phosphorothioate-modified at 3' internucleotide bond
  modified_base (10)..(17): phosphorothioate-modified at 3' internucleotide bond
  modified_base (19)..(26): phosphorothioate-modified at 3' internucleotide bond
  modified_base (28)..(35): phosphorothioate-modified at 3' internucleotide bond
ctcctcctcctcctcctcctcctcctcctcctcctc

SEQ ID NO: 34 - DNA, 36 bp, Artificial Sequence; identical to SEQ ID NO: 33
  Inhibitory Oligonucleotide
  modified_base (1)..(5): phosphorothioate-modified at 3' internucleotide bond
  modified_base (7)..(14): phosphorothioate-modified at 3' internucleotide bond
  modified_base (16)..(23): phosphorothioate-modified at 3' internucleotide bond
  modified_base (25)..(32): phosphorothioate-modified at 3' internucleotide bond
  modified_base (34)..(35): phosphorothioate-modified at 3' internucleotide bond

SEQ ID NO: 35 - DNA, 36 bp, Artificial Sequence; identical to SEQ ID NO: 33
  Inhibitory Oligonucleotide
  modified_base (1)..(2): phosphorothioate-modified at 3' internucleotide bond
  modified_base (4)..(11): phosphorothioate-modified at 3' internucleotide bond
  modified_base (13)..(20): phosphorothioate-modified at 3' internucleotide bond
  modified_base (22)..(29): phosphorothioate-modified at 3' internucleotide bond
  modified_base (31)..(35): phosphorothioate-modified at 3' internucleotide bond

SEQ ID NO: 36 - DNA, 18 bp, Artificial Sequence
  Inhibitory Oligonucleotide
  modified_base (1)..(8): phosphorothioate-modified at 3' internucleotide bond
  modified_base (10)..(17): phosphorothioate-modified at 3' internucleotide bond
tcctcctcctcctcctcc

SEQ ID NO: 37 - DNA, 27 bp, Artificial Sequence
  Inhibitory Oligonucleotide
  modified_base (1)..(8): phosphorothioate-modified at 3' internucleotide bond
  modified_base (10)..(17): phosphorothioate-modified at 3' internucleotide bond
  modified_base (19)..(26): phosphorothioate-modified at 3' internucleotide bond
tcctcctcctcctcctcctcctcctcc

SEQ ID NO: 38 - DNA, 27 bp, Artificial Sequence
  Inhibitory Oligonucleotide
  modified_base (1)..(5): phosphorothioate-modified at 3' internucleotide bond
  modified_base (7)..(14): phosphorothioate-modified at 3' internucleotide bond
  modified_base (16)..(23): phosphorothioate-modified at 3' internucleotide bond
  modified_base (25)..(26): phosphorothioate-modified at 3' internucleotide bond
tcctcctcctcctcctcctcctcctcc

SEQ ID NO: 39 - DNA, 27 bp, Artificial Sequence
  Inhibitory Oligonucleotide
  modified_base (1)..(2): phosphorothioate-modified at 3' internucleotide bond
  modified_base (4)..(11): phosphorothioate-modified at 3' internucleotide bond
  modified_base (13)..(20): phosphorothioate-modified at 3' internucleotide bond
  modified_base (22)..(26): phosphorothioate-modified at 3' internucleotide bond
tcctcctcctcctcctcctcctcctcc

SEQ ID NO: 40 - DNA, 36 bp, Artificial Sequence; identical to SEQ ID NO: 20
  Inhibitory Oligonucleotide
  modified_base (1)..(8): phosphorothioate-modified at 3' internucleotide bond
  modified_base (10)..(17): phosphorothioate-modified at 3' internucleotide bond
  modified_base (19)..(26): phosphorothioate-modified at 3' internucleotide bond
  modified_base (28)..(35): phosphorothioate-modified at 3' internucleotide bond

SEQ ID NO: 41 - DNA, 36 bp, Artificial Sequence; identical to SEQ ID NO: 20
  Inhibitory Oligonucleotide
  modified_base (1)..(5): phosphorothioate-modified at 3' internucleotide bond
  modified_base (7)..(14): phosphorothioate-modified at 3' internucleotide bond
  modified_base (16)..(23): phosphorothioate-modified at 3' internucleotide bond
  modified_base (25)..(32): phosphorothioate-modified at 3' internucleotide bond
  modified_base (34)..(35): phosphorothioate-modified at 3' internucleotide bond

SEQ ID NO: 42 - DNA, 36 bp, Artificial Sequence; identical to SEQ ID NO: 20
  Inhibitory Oligonucleotide
  modified_base (1)..(2): phosphorothioate-modified at 3' internucleotide bond
  modified_base (4)..(11): phosphorothioate-modified at 3' internucleotide bond
  modified_base (13)..(20): phosphorothioate-modified at 3' internucleotide bond
  modified_base (22)..(29): phosphorothioate-modified at 3' internucleotide bond
  modified_base (31)..(35): phosphorothioate-modified at 3' internucleotide bond

SEQ ID NO: 43 - DNA, 22 bp, Artificial Sequence
  CpG2395 TLR9 stimulatory oligonucleotide
  modified_base (1)..(21): phosphorothioate-modified at 3' internucleotide bond
tcgtcgttttcggcgcgcgccg

SEQ ID NO: 44 - DNA, 20 bp, Artificial Sequence
  CpG2216 stimulatory oligonucleotide
  modified_base (1)..(2): phosphorothioate-modified at 3' internucleotide bond
  modified_base (15)..(19): phosphorothioate-modified at 3' internucleotide bond
gggggacgatcgtcgggggg

SEQ ID NO: 45 - DNA, 18 bp, Artificial Sequence
  Inhibitory oligonucleotide
  modified_base (1)..(17): phosphorothioate-modified at 3' internucleotide bond
cctcctcctcctcctcct

SEQ ID NO: 46 - DNA, 36 bp, Artificial Sequence; identical to SEQ ID NO: 15
  Inhibitory Oligonucleotide
  modified_base (1)..(35): phosphorothioate-modified at 3' internucleotide bond

SEQ ID NO: 47 - DNA, 36 bp, Artificial Sequence; identical to SEQ ID NO: 15
  Inhibitory Oligonucleotide
  modified_base (1)..(5): phosphorothioate-modified at 3' internucleotide bond
  modified_base (7)..(17): phosphorothioate-modified at 3' internucleotide bond
  modified_base (19)..(29): phosphorothioate-modified at 3' internucleotide bond
  modified_base (31)..(35): phosphorothioate-modified at 3' internucleotide bond

SEQ ID NO: 48 - DNA, 36 bp, Artificial Sequence; identical to SEQ ID NO: 15
  Inhibitory Oligonucleotide
  modified_base (1)..(2): phosphorothioate-modified at 3' internucleotide bond
  modified_base (4)..(8): phosphorothioate-modified at 3' internucleotide bond
  modified_base (10)..(20): phosphorothioate-modified at 3' internucleotide bond
  modified_base (22)..(32): phosphorothioate-modified at 3' internucleotide bond
  modified_base (34)..(35): phosphorothioate-modified at 3' internucleotide bond

SEQ ID NO: 49 - DNA, 36 bp, Artificial Sequence; identical to SEQ ID NO: 20
  Inhibitory Oligonucleotide
  modified_base (1)..(35): phosphorothioate-modified at 3' internucleotide bond

SEQ ID NO: 50 - DNA, 36 bp, Artificial Sequence; identical to SEQ ID NO: 20
  Inhibitory Oligonucleotide
  modified_base (1)..(5): phosphorothioate-modified at 3' internucleotide bond
  modified_base (7)..(17): phosphorothioate-modified at 3' internucleotide bond
  modified_base (19)..(29): phosphorothioate-modified at 3' internucleotide bond
  modified_base (31)..(35): phosphorothioate-modified at 3' internucleotide bond